European Patent Specification EP 3 658 154 B1, published July 10, 2024. Title: Antisense drugs against canine ICAM-1. Applicant: Universität zu Lübeck. The sequence listing filed with the application follows.

SEQUENCE LISTING (15 sequences)

SEQ ID NO: 1 - DNA, 18 bp, Artificial sequence
  Antisense oligonucleotide
tcttccgctggcggttat

SEQ ID NO: 2 - DNA, 18 bp, Artificial sequence
  Antisense oligonucleotide
ccgctggcggttatagag

SEQ ID NO: 3 - DNA, 18 bp, Artificial sequence
  Antisense oligonucleotide
atcttccgctggcggtta

SEQ ID NO: 4 - DNA, 18 bp, Artificial sequence
  Scrambled negative control oligonucleotide
caggtggtcagatggacc

SEQ ID NO: 5 - DNA, 24 bp, Artificial sequence
  Primer sequence
tgacaaccattgtcatcttaggaa

SEQ ID NO: 6 - DNA, 20 bp, Artificial sequence
  Primer sequence
ggtgtgttcagcttcatggc

SEQ ID NO: 7 - DNA, 21 bp, Artificial sequence
  Primer sequence
cacatccaaggaaggcagcag

SEQ ID NO: 8 - DNA, 21 bp, Artificial sequence
  Primer sequence
gacttgccctccaatggatcc

SEQ ID NO: 9 - DNA, 25 bp, Artificial sequence
  Primer sequence
gccacttcttctgtaagtctgtggg

SEQ ID NO: 10 - DNA, 17 bp, Artificial sequence
  Primer sequence
ctaccggccctgggacg

SEQ ID NO: 11 - DNA, 20 bp, Artificial sequence
  Primer sequence
aacagcgacacccactcctc

SEQ ID NO: 12 - DNA, 21 bp, Artificial sequence
  Primer sequence
ggaggggagattcagtgtggt

SEQ ID NO: 13 - DNA, 51 bp, Canis lupus familiaris
tgtagccgcttacctctataaccgccagcggaagatccagaaatacaagct

SEQ ID NO: 14 - DNA, 21 bp, Artificial sequence
  strand of si1559a
cucuauaaccgccagcggatt

SEQ ID NO: 15 - DNA, 21 bp, Artificial sequence
  strand of si1559a
uccgcuggcgguuauagagtt